European Patent Specification EP 3 645 011 B1, published October 4, 2023. Title: Method for preparing GOS having reduced allergenicity. Applicant: FrieslandCampina Nederland B.V. The sequence listing filed with the application follows.

SEQUENCE LISTING (16 sequences)

SEQ ID NO: 1 - protein, 696 aa, Cryptococcus terrestris
MIPASALLAAVPLLAQQVSAGILRRQNAAGSDSAAPDSIADASTGVVSSIATEAVSSGATGLVASVAMSFASSMATPTATVTGLSSETGAPSNTPMASASGSVPTTTSAVGSGDFDWVQTDGLPTITTTLATTNQDAITPTATGPVGGQGTPAVNFTDYSSSSLEQFWNDWVGEVEEPPFAYVPEPPNPYPLPNAPPPIYPEYYTKRPKDILPDYKFPKDFLFGWATAAQQWEGAVKADGKGPSIWDWASRFPGFIADNTTSDVGDLGYYLYKEDLARIAALGANVYSFSMFWTRIFPFGKADSPVNQAGIDFYHDLIDYSWSLGIEPVVTLFHWDTPLALQLEYGGFASERIIDDYVNYAETVFKAYNGSVHKWVTFNEPVVFCSQMAAPVNTTLPPNLNSTIYPYTCSYHLVLAHAKTVKRFRELNIQGQIAFKSDNFVGIPWREGNQEDIDAVERHQAYQIGIFAEPIYNTGDWPDIVKNDLSPDILPRFTDDEIAMIKCTADFFPIDGYRDGYVQAVPGGVEACVANISNPLWPACNQVNFYDSTPAGWAIGTFGNWPTTPWLQNTWQFVRPFLADLAKRYPTEGGIYLSEFGFSEPFENDKTFIYQITQDSGRTAYFNSYLGEVLKGIVEDGIPIKGVFGWSMVDNFEWNSGLSTRFGVQYVDYNSPTRQRTFKRSALEMSEFWNAHRCSA

SEQ ID NO: 2 - protein, 566 aa, Cryptococcus terrestris
ATTNQDAITPTATGPVGGQGTPAVNFTDYSSSSLEQFWNDWVGEVEEPPFAYVPEPPNPYPLPNAPPPIYPEYYTKRPKDILPDYKFPKDFLFGWATAAQQWEGAVKADGKGPSIWDWASRFPGFIADNTTSDVGDLGYYLYKEDLARIAALGANVYSFSMFWTRIFPFGKADSPVNQAGIDFYHDLIDYSWSLGIEPVVTLFHWDTPLALQLEYGGFASERIIDDYVNYAETVFKAYNGSVHKWVTFNEPVVFCSQMAAPVNTTLPPNLNSTIYPYTCSYHLVLAHAKTVKRFRELNIQGQIAFKSDNFVGIPWREGNQEDIDAVERHQAYQIGIFAEPIYNTGDWPDIVKNDLSPDILPRFTDDEIAMIKCTADFFPIDGYRDGYVQAVPGGVEACVANISNPLWPACNQVNFYDSTPAGWAIGTFGNWPTTPWLQNTWQFVRPFLADLAKRYPTEGGIYLSEFGFSEPFENDKTFIYQITQDSGRTAYFNSYLGEVLKGIVEDGIPIKGVFGWSMVDNFEWNSGLSTRFGVQYVDYNSPTRQRTFKRSALEMSEFWNAHRCSA

SEQ ID NO: 3 - protein, 560 aa, Cryptococcus terrestris
AITPTATGPVGGQGTPAVNFTDYSSSSLEQFWNDWVGEVEEPPFAYVPEPPNPYPLPNAPPPIYPEYYTKRPKDILPDYKFPKDFLFGWATAAQQWEGAVKADGKGPSIWDWASRFPGFIADNTTSDVGDLGYYLYKEDLARIAALGANVYSFSMFWTRIFPFGKADSPVNQAGIDFYHDLIDYSWSLGIEPVVTLFHWDTPLALQLEYGGFASERIIDDYVNYAETVFKAYNGSVHKWVTFNEPVVFCSQMAAPVNTTLPPNLNSTIYPYTCSYHLVLAHAKTVKRFRELNIQGQIAFKSDNFVGIPWREGNQEDIDAVERHQAYQIGIFAEPIYNTGDWPDIVKNDLSPDILPRFTDDEIAMIKCTADFFPIDGYRDGYVQAVPGGVEACVANISNPLWPACNQVNFYDSTPAGWAIGTFGNWPTTPWLQNTWQFVRPFLADLAKRYPTEGGIYLSEFGFSEPFENDKTFIYQITQDSGRTAYFNSYLGEVLKGIVEDGIPIKGVFGWSMVDNFEWNSGLSTRFGVQYVDYNSPTRQRTFKRSALEMSEFWNAHRCSA

SEQ ID NO: 4 - protein, 555 aa, Cryptococcus terrestris
ATGPVGGQGTPAVNFTDYSSSSLEQFWNDWVGEVEEPPFAYVPEPPNPYPLPNAPPPIYPEYYTKRPKDILPDYKFPKDFLFGWATAAQQWEGAVKADGKGPSIWDWASRFPGFIADNTTSDVGDLGYYLYKEDLARIAALGANVYSFSMFWTRIFPFGKADSPVNQAGIDFYHDLIDYSWSLGIEPVVTLFHWDTPLALQLEYGGFASERIIDDYVNYAETVFKAYNGSVHKWVTFNEPVVFCSQMAAPVNTTLPPNLNSTIYPYTCSYHLVLAHAKTVKRFRELNIQGQIAFKSDNFVGIPWREGNQEDIDAVERHQAYQIGIFAEPIYNTGDWPDIVKNDLSPDILPRFTDDEIAMIKCTADFFPIDGYRDGYVQAVPGGVEACVANISNPLWPACNQVNFYDSTPAGWAIGTFGNWPTTPWLQNTWQFVRPFLADLAKRYPTEGGIYLSEFGFSEPFENDKTFIYQITQDSGRTAYFNSYLGEVLKGIVEDGIPIKGVFGWSMVDNFEWNSGLSTRFGVQYVDYNSPTRQRTFKRSALEMSEFWNAHRCSA

SEQ ID NO: 5 - DNA, 2091 bp, Cryptococcus terrestris
atgatcccggcaagtgcactccttgccgccgtacccctccttgcccaacaggtgagcgccggcatactgcgaagacagaatgctgcgggttcggattcggcagcgcctgactcgatcgcggatgcgtccaccggtgtcgtctcgtcgatcgccacggaagccgtctcttcgggagcgacaggccttgtcgcgtccgtcgccatgtcattcgcctcgtcgatggcgactccaacggccacagtgacgggcctaagctccgagacgggagcgccttccaacaccccaatggccagtgcctctggtagtgtccctacaaccacctctgccgtcgggtctggcgacttcgactgggtccagacagacggcctgcccacgatcacgaccactttggctactacgaaccaggacgcaatcactccgacggcgacgggccccgtcggcggacagggcacccctgctgtcaacttcaccgactactcttcatcgtcgctcgagcagttttggaacgactgggtgggagaggtggaggagccgccgttcgcctacgtcccggaaccgcctaacccgtacccgttaccgaacgccccgcctccaatctaccccgagtactacaccaagcgtcccaaggacattctccccgactacaagttccccaaagacttcctgtttggctgggcgaccgccgcgcagcagtgggagggggccgtcaaggcggatgggaaggggccgtccatctgggactgggccagccggttcccggggttcattgcggacaacacgacttccgacgtcggagacttgggatactatttatacaaagaggacctcgctaggatcgctgcattgggcgcaaacgtttactctttcagcatgttctggacacggatctttcccttcggcaaggccgactcgcctgtcaatcaagcgggcatcgacttctaccacgacttgatcgattattcttggagcctgggcatcgagcccgtcgtgacattgttccattgggatacgccgctcgccctccagcttgagtacggaggtttcgccagcgagcgaatcattgatgactacgtcaactatgcggaaaccgtgttcaaggcgtacaacggtagtgtgcacaaatgggtcacattcaacgagcctgtggtgttctgcagccagatggcagcgcccgtgaacactactctaccgccgaacctcaactcgacaatctacccctatacctgcagctatcacctcgtgctagcccacgccaagacggtcaagcggttcagggagttgaacattcagggccagatcgctttcaagtcggacaattttgtcggtatcccgtggcgtgaggggaaccaagaggacatagatgcggtcgagcgccatcaggcgtaccagatcgggatctttgctgagccgatctacaacaccggagactggcccgatatcgtgaagaatgatctctcccccgacatccttcctcgattcacggatgacgagatcgcgatgatcaagtgcactgccgacttcttccccatcgatggctacagggacggttatgtccaggctgtaccggggggtgtcgaagcttgcgtcgcgaacatcagcaacccgctttggcctgcttgcaaccaagtcaacttctatgattccacacccgccggatgggcgatcggcacgttcggcaactggccgacgacaccctggctccagaacacctggcagtttgtgcgccccttcctcgctgatctggcaaagcggtaccccaccgaaggcggcatctacctttcggaatttggcttctccgagccgttcgaaaatgataaaaccttcatttaccagatcacccaggacagcggacggacggcgtacttcaacagttacctcggcgaagtgttgaaaggtatcgttgaagatggcattcctatcaagggcgtgttcggctggagtatggtcgacaactttgaatggaactctggcttgtctactcgcttcggcgtccaatacgttgattacaacagcccgacgcgtcaacgaacgttcaagcggtccgctctggagatgagcgagttctggaatgctcatcgatgttccgcctaa

SEQ ID NO: 6 - DNA, 1701 bp, Cryptococcus terrestris
gctactacgaaccaggacgcaatcactccgacggcgacgggccccgtcggcggacagggcacccctgctgtcaacttcaccgactactcttcatcgtcgctcgagcagttttggaacgactgggtgggagaggtggaggagccgccgttcgcctacgtcccggaaccgcctaacccgtacccgttaccgaacgccccgcctccaatctaccccgagtactacaccaagcgtcccaaggacattctccccgactacaagttccccaaagacttcctgtttggctgggcgaccgccgcgcagcagtgggagggggccgtcaaggcggatgggaaggggccgtccatctgggactgggccagccggttcccggggttcattgcggacaacacgacttccgacgtcggagacttgggatactatttatacaaagaggacctcgctaggatcgctgcattgggcgcaaacgtttactctttcagcatgttctggacacggatctttcccttcggcaaggccgactcgcctgtcaatcaagcgggcatcgacttctaccacgacttgatcgattattcttggagcctgggcatcgagcccgtcgtgacattgttccattgggatacgccgctcgccctccagcttgagtacggaggtttcgccagcgagcgaatcattgatgactacgtcaactatgcggaaaccgtgttcaaggcgtacaacggtagtgtgcacaaatgggtcacattcaacgagcctgtggtgttctgcagccagatggcagcgcccgtgaacactactctaccgccgaacctcaactcgacaatctacccctatacctgcagctatcacctcgtgctagcccacgccaagacggtcaagcggttcagggagttgaacattcagggccagatcgctttcaagtcggacaattttgtcggtatcccgtggcgtgaggggaaccaagaggacatagatgcggtcgagcgccatcaggcgtaccagatcgggatctttgctgagccgatctacaacaccggagactggcccgatatcgtgaagaatgatctctcccccgacatccttcctcgattcacggatgacgagatcgcgatgatcaagtgcactgccgacttcttccccatcgatggctacagggacggttatgtccaggctgtaccggggggtgtcgaagcttgcgtcgcgaacatcagcaacccgctttggcctgcttgcaaccaagtcaacttctatgattccacacccgccggatgggcgatcggcacgttcggcaactggccgacgacaccctggctccagaacacctggcagtttgtgcgccccttcctcgctgatctggcaaagcggtaccccaccgaaggcggcatctacctttcggaatttggcttctccgagccgttcgaaaatgataaaaccttcatttaccagatcacccaggacagcggacggacggcgtacttcaacagttacctcggcgaagtgttgaaaggtatcgttgaagatggcattcctatcaagggcgtgttcggctggagtatggtcgacaactttgaatggaactctggcttgtctactcgcttcggcgtccaatacgttgattacaacagcccgacgcgtcaacgaacgttcaagcggtccgctctggagatgagcgagttctggaatgctcatcgatgttccgcctaa

SEQ ID NO: 7 - DNA, 1683 bp, Cryptococcus terrestris
gcaatcactccgacggcgacgggccccgtcggcggacagggcacccctgctgtcaacttcaccgactactcttcatcgtcgctcgagcagttttggaacgactgggtgggagaggtggaggagccgccgttcgcctacgtcccggaaccgcctaacccgtacccgttaccgaacgccccgcctccaatctaccccgagtactacaccaagcgtcccaaggacattctccccgactacaagttccccaaagacttcctgtttggctgggcgaccgccgcgcagcagtgggagggggccgtcaaggcggatgggaaggggccgtccatctgggactgggccagccggttcccggggttcattgcggacaacacgacttccgacgtcggagacttgggatactatttatacaaagaggacctcgctaggatcgctgcattgggcgcaaacgtttactctttcagcatgttctggacacggatctttcccttcggcaaggccgactcgcctgtcaatcaagcgggcatcgacttctaccacgacttgatcgattattcttggagcctgggcatcgagcccgtcgtgacattgttccattgggatacgccgctcgccctccagcttgagtacggaggtttcgccagcgagcgaatcattgatgactacgtcaactatgcggaaaccgtgttcaaggcgtacaacggtagtgtgcacaaatgggtcacattcaacgagcctgtggtgttctgcagccagatggcagcgcccgtgaacactactctaccgccgaacctcaactcgacaatctacccctatacctgcagctatcacctcgtgctagcccacgccaagacggtcaagcggttcagggagttgaacattcagggccagatcgctttcaagtcggacaattttgtcggtatcccgtggcgtgaggggaaccaagaggacatagatgcggtcgagcgccatcaggcgtaccagatcgggatctttgctgagccgatctacaacaccggagactggcccgatatcgtgaagaatgatctctcccccgacatccttcctcgattcacggatgacgagatcgcgatgatcaagtgcactgccgacttcttccccatcgatggctacagggacggttatgtccaggctgtaccggggggtgtcgaagcttgcgtcgcgaacatcagcaacccgctttggcctgcttgcaaccaagtcaacttctatgattccacacccgccggatgggcgatcggcacgttcggcaactggccgacgacaccctggctccagaacacctggcagtttgtgcgccccttcctcgctgatctggcaaagcggtaccccaccgaaggcggcatctacctttcggaatttggcttctccgagccgttcgaaaatgataaaaccttcatttaccagatcacccaggacagcggacggacggcgtacttcaacagttacctcggcgaagtgttgaaaggtatcgttgaagatggcattcctatcaagggcgtgttcggctggagtatggtcgacaactttgaatggaactctggcttgtctactcgcttcggcgtccaatacgttgattacaacagcccgacgcgtcaacgaacgttcaagcggtccgctctggagatgagcgagttctggaatgctcatcgatgttccgcctaa

SEQ ID NO: 8 - DNA, 1668 bp, Cryptococcus terrestris
gcgacgggccccgtcggcggacagggcacccctgctgtcaacttcaccgactactcttcatcgtcgctcgagcagttttggaacgactgggtgggagaggtggaggagccgccgttcgcctacgtcccggaaccgcctaacccgtacccgttaccgaacgccccgcctccaatctaccccgagtactacaccaagcgtcccaaggacattctccccgactacaagttccccaaagacttcctgtttggctgggcgaccgccgcgcagcagtgggagggggccgtcaaggcggatgggaaggggccgtccatctgggactgggccagccggttcccggggttcattgcggacaacacgacttccgacgtcggagacttgggatactatttatacaaagaggacctcgctaggatcgctgcattgggcgcaaacgtttactctttcagcatgttctggacacggatctttcccttcggcaaggccgactcgcctgtcaatcaagcgggcatcgacttctaccacgacttgatcgattattcttggagcctgggcatcgagcccgtcgtgacattgttccattgggatacgccgctcgccctccagcttgagtacggaggtttcgccagcgagcgaatcattgatgactacgtcaactatgcggaaaccgtgttcaaggcgtacaacggtagtgtgcacaaatgggtcacattcaacgagcctgtggtgttctgcagccagatggcagcgcccgtgaacactactctaccgccgaacctcaactcgacaatctacccctatacctgcagctatcacctcgtgctagcccacgccaagacggtcaagcggttcagggagttgaacattcagggccagatcgctttcaagtcggacaattttgtcggtatcccgtggcgtgaggggaaccaagaggacatagatgcggtcgagcgccatcaggcgtaccagatcgggatctttgctgagccgatctacaacaccggagactggcccgatatcgtgaagaatgatctctcccccgacatccttcctcgattcacggatgacgagatcgcgatgatcaagtgcactgccgacttcttccccatcgatggctacagggacggttatgtccaggctgtaccggggggtgtcgaagcttgcgtcgcgaacatcagcaacccgctttggcctgcttgcaaccaagtcaacttctatgattccacacccgccggatgggcgatcggcacgttcggcaactggccgacgacaccctggctccagaacacctggcagtttgtgcgccccttcctcgctgatctggcaaagcggtaccccaccgaaggcggcatctacctttcggaatttggcttctccgagccgttcgaaaatgataaaaccttcatttaccagatcacccaggacagcggacggacggcgtacttcaacagttacctcggcgaagtgttgaaaggtatcgttgaagatggcattcctatcaagggcgtgttcggctggagtatggtcgacaactttgaatggaactctggcttgtctactcgcttcggcgtccaatacgttgattacaacagcccgacgcgtcaacgaacgttcaagcggtccgctctggagatgagcgagttctggaatgctcatcgatgttccgcctaa

SEQ ID NO: 9 - protein, 11 aa, Cryptococcus terrestris
GVQYVDYNSPT

SEQ ID NO: 10 - protein, 11 aa, Cryptococcus terrestris
FLFGWATAAQQ

SEQ ID NO: 11 - protein, 15 aa, Cryptococcus terrestris
QAYQIGIFAEPIYNT

SEQ ID NO: 12 - protein, 8 aa, Cryptococcus terrestris
PSIWDWAS

SEQ ID NO: 13 - protein, 10 aa, Cryptococcus terrestris
EEPPFAYVPE

SEQ ID NO: 14 - DNA, 41 bp, Artificial Sequence
  5'RACE GSP primer
gattacgccaagcttgcaaagatcccgatctggtacgcctg

SEQ ID NO: 15 - DNA, 39 bp, Artificial Sequence
  3'RACE GSP primer
gattacgccaagcttttcctgtttggctgggcgaccgcc

SEQ ID NO: 16 - DNA, 2942 bp, Cryptococcus terrestris
atgatcccggcaagtgcactccttgccgccgtacccctccttgcccaacaggtgagcgccggcatactgcgaagacagaatgctgcgggttcggattcggcagcgcctgactcgatcgcggatgcgtccaccggtgtcgtctcgtcgatcgccacggaagccgtctcttcgggagcgacaggccttgtcgcgtccgtcgccatgtcattcgcctcgtcgatggcgactccaacggccacagtgacgggcctaagctccgagacgggagcgccttccaacaccccaatggccagtgcctctggtagtgtccctacaaccacctctgccgtcgggtctggcgacttcgactgggtccagacagacggcctgcccacgatcacgaccactttggctactacgaaccaggacgcaatcactccgacggcgacgggccccgtcggcggacagggcacccctgctgtcaacttcaccgactactcttcatcgtcgctcgagcagttttggaacgactgggtaagttaggccacggctccatctgctgacgagggtccaggagagctgacgcacaggtgggagaggtggaggagccgccgttcgcctacgtcccggaaccgcctaacccgtacccgttaccgaacgccccgcctccaatctaccccgagtactacaccaagcgtcccaaggacattctccccgactacaagttccccaaagacttcctgtttggctgggcgaccgccgcgcagcagtgggagggggccgtcaaggcggatgggaaggggccgtccatctgggactgggccagccggttcccggggttcattgcggacaacacgacttccggtgagctgagaatgaccacctttcagtacgagagctcacttcagacgtcggagacttgggatactatttatacaaagagggttagccggggccgtatgagccagtgctggatgctgagtgcagacctcgctaggatcgctgcattgggcgcaaacgtttactctttcagcatgttctggacacggatctttcccttcggcaaggccgactcgcctgtcaatcaagcgggcatcgacttctaccacgacttgatcgattattcttggagcctgggcatcgagcccgtcgtgtaagcctgtacaggggcccatcttgaaccccgctcattacaggacattgttccattgggatacgccgctcgccctccagcttgagtacggaggtttcgccagcgagcgaatcattgatgactacgtcaactatgcggtgagcagtacggtcccttgagcacagcttgggctgactcgtaaggaaaccgtgttcaaggcgtacaacggtagtgtgcacaaatgggtcacattcaacgagcctgtggtgttctgcagccaggtgagcaaccaaagcgcatgttgagctgatcgaccagatggcagcgcccgtgaacgtaagatgagcaacgagccagaccagtgtcaatgctgaccatgaccgtagactactctaccgccgaacctcaactcgacaatctacccctatacctgcagctatcacctcgtgctagcccacgccaagacggtcaagcggttcagggagttgaacattcgtgagctgatcggtaccgcgtttctggctgaagacacgctgactgtcacagagggccagatcgctttcaagtcggacaattttgtgtgagcatcgctgttgtggggagtcgtgcgtgctgaacctttagcggtatcccgtggcgtgaggggaaccaagaggacatagatgcggtcgagcgccatcaggtgaagtctcgccagaccgcggaggctccgaggctgaccggacaggcgtaccagatcgggatctttgctgagccgatctacaacaccggagtgaggcttccctccctcttccgcacggtacacttgtggcttatcgacaggactggcccgatatcgtgaagaatgatctctcccccgacatccttcctcgattcacggatgacgagatcgcgatgatcaagtgcactgccgacttcttccccatcgatgtgagcctccaaacccacccgtcgggagacgggtcccgagtactacgcctaacgcacagggctacagggacggttatgtccaggctgtaccggggggtgtcgaagcttgcgtcgcgaacatcagcaacccgctttggcctgcttgcaaccaagtcaagtgagactcgtccagaccccgcctgtattgcgagcgccggcactgacatgcagcttctgtacggcccacagcaccccgtcgccgccgctgagctgatgcatagatgattccacacccgccggatgggcgatcggcacgttcggcaactggccgacgacaccctggctccagaacacctggcagtttgtgcgccccttcctcgctgatctggcaaagcggtaccccaccgaaggcggcatctacctttcggaatttggcttctccgagccgttcgaaaatgagtacgcctatcaactggctgctgcaaggcatggcgtactgagactcagtaaaaccttcatttaccagatcacccaggacagcggacggacggcgtacttcaacagttacctcggcgaagtgttgaaaggtatcgttgaagatggcattcctatcaagggcgtgttcggctggagtatggtcgacaactttgaatggaactctggcttgtctagtacgtccacacggccgtggatccttcgacgcccggtctgacccgtagctcgcttcggcgtccaatacgttgattacaacaggtgagctgtcgtttttgttttagggatcgcgatgctgatgcaaacagcccgacgcgtcaacgaacggtacgccgttcatgacctccccctcgtccctgctgacgtccagttcaagcggtccgctctggagatgagcgagttctggaatgctcatcgatgttccgcctaa